European Patent Specification EP 4 015 648 B1, published November 13, 2024. Title: Reducing Intron Retention. Applicant: University of Southampton. The sequence listing filed with the application follows.

SEQUENCE LISTING (473 sequences)

SEQ ID NO: 1 - RNA, 18 nt, Artificial Sequence
  SSO
cugcagagcuggggccug

SEQ ID NO: 2 - DNA, 18 bp, Artificial Sequence
  SSO
ctgcagagctggggcctg

SEQ ID NO: 3 - RNA, 18 nt, Homo sapiens
caggccccagcucugcag

SEQ ID NO: 4 - RNA, 16 nt, Artificial Sequence
  SSO
ugcagagcuggggccu

SEQ ID NO: 5 - DNA, 16 bp, Artificial Sequence
  SSO
tgcagagctggggcct

SEQ ID NO: 6 - RNA, 16 nt, Homo sapiens
aggccccagcucugca

SEQ ID NO: 7 - RNA, 16 nt, Artificial Sequence
  SSO
gcagagcuggggccug

SEQ ID NO: 8 - DNA, 16 bp, Artificial Sequence
  SSO
gcagagctggggcctg

SEQ ID NO: 9 - RNA, 16 nt, Homo sapiens
caggccccagcucugc

SEQ ID NO: 10 - RNA, 16 nt, Artificial Sequence
  SSO
cagagcuggggccugg

SEQ ID NO: 11 - DNA, 16 bp, Artificial Sequence
  SSO
cagagctggggcctgg

SEQ ID NO: 12 - RNA, 16 nt, Homo sapiens
ccaggccccagcucug

SEQ ID NO: 13 - RNA, 16 nt, Artificial Sequence
  SSO
agagcuggggccuggg

SEQ ID NO: 14 - DNA, 16 bp, Artificial Sequence
  SSO
agagctggggcctggg

SEQ ID NO: 15 - RNA, 16 nt, Homo sapiens
cccaggccccagcucu

SEQ ID NO: 16 - RNA, 16 nt, Artificial Sequence
  SSO
gagcuggggccugggg

SEQ ID NO: 17 - DNA, 16 bp, Artificial Sequence
  SSO
gagctggggcctgggg

SEQ ID NO: 18 - RNA, 16 nt, Homo sapiens
ccccaggccccagcuc

SEQ ID NO: 19 - RNA, 16 nt, Artificial Sequence
  SSO
agcuggggccuggggu

SEQ ID NO: 20 - DNA, 16 bp, Artificial Sequence
  SSO
agctggggcctggggt

SEQ ID NO: 21 - RNA, 16 nt, Homo sapiens
accccaggccccagcu

SEQ ID NO: 22 - RNA, 16 nt, Artificial Sequence
  SSO
gcuggggccugggguc

SEQ ID NO: 23 - DNA, 16 bp, Artificial Sequence
  SSO
gctggggcctggggtc

SEQ ID NO: 24 - RNA, 16 nt, Homo sapiens
gaccccaggccccagc

SEQ ID NO: 25 - RNA, 16 nt, Artificial Sequence
  SSO
cuggggccuggggucc

SEQ ID NO: 26 - DNA, 16 bp, Artificial Sequence
  SSO
ctggggcctggggtcc

SEQ ID NO: 27 - RNA, 16 nt, Homo sapiens
ggaccccaggccccag

SEQ ID NO: 28 - RNA, 16 nt, Artificial Sequence
  SSO
uggggccuggggucca

SEQ ID NO: 29 - DNA, 16 bp, Artificial Sequence
  SSO
tggggcctggggtcca

SEQ ID NO: 30 - RNA, 16 nt, Homo sapiens
uggaccccaggcccca

SEQ ID NO: 31 - RNA, 16 nt, Artificial Sequence
  SSO
ggggccugggguccag

SEQ ID NO: 32 - DNA, 16 bp, Artificial Sequence
  SSO
ggggcctggggtccag

SEQ ID NO: 33 - RNA, 16 nt, Homo sapiens
cuggaccccaggcccc

SEQ ID NO: 34 - RNA, 16 nt, Artificial Sequence
  SSO
cugcagagcuggggcc

SEQ ID NO: 35 - DNA, 16 bp, Artificial Sequence
  SSO
ctgcagagctggggcc

SEQ ID NO: 36 - RNA, 16 nt, Homo sapiens
ggccccagcucugcag

SEQ ID NO: 37 - RNA, 16 nt, Artificial Sequence
  SSO
gcugcagagcuggggc

SEQ ID NO: 38 - DNA, 16 bp, Artificial Sequence
  SSO
gctgcagagctggggc

SEQ ID NO: 39 - RNA, 16 nt, Homo sapiens
gccccagcucugcagc

SEQ ID NO: 40 - RNA, 16 nt, Artificial Sequence
  SSO
ugcugcagagcugggg

SEQ ID NO: 41 - DNA, 16 bp, Artificial Sequence
  SSO
tgctgcagagctgggg

SEQ ID NO: 42 - RNA, 16 nt, Homo sapiens
ccccagcucugcagca

SEQ ID NO: 43 - RNA, 16 nt, Artificial Sequence
  SSO
cugcugcagagcuggg

SEQ ID NO: 44 - DNA, 16 bp, Artificial Sequence
  SSO
ctgctgcagagctggg

SEQ ID NO: 45 - RNA, 16 nt, Homo sapiens
cccagcucugcagcag

SEQ ID NO: 46 - RNA, 29 nt, Homo sapiens
cuggaccccaggccccagcucugcagcag

SEQ ID NO: 47 - RNA, 26 nt, Homo sapiens
uagagaggugugggaagggaagcaga

SEQ ID NO: 48 - RNA, 38 nt, Homo sapiens
aauuccuucaucauggcacauuuauccuugcagacagg

SEQ ID NO: 49 - RNA, 28 nt, Homo sapiens
ccugaggauacucacagaaaggcaacag

SEQ ID NO: 50 - RNA, 21 nt, Homo sapiens
uuuccccaacacacuccagca

SEQ ID NO: 51 - RNA, 18 nt, Homo sapiens
gggccgcugcccaccguc

SEQ ID NO: 52 - RNA, 22 nt, Homo sapiens
cagcacagcucagaagucugag

SEQ ID NO: 53 - RNA, 28 nt, Homo sapiens
ccaagccagggacagggaggugaaugcc

SEQ ID NO: 54 - RNA, 22 nt, Homo sapiens
cuucugcccagcucucugacug

SEQ ID NO: 55 - RNA, 26 nt, Homo sapiens
ucuucacaaaccccugcaaaaaugag

SEQ ID NO: 56 - RNA, 24 nt, Homo sapiens
cccaaagcccccgcaggugcagcc

SEQ ID NO: 57 - RNA, 21 nt, Homo sapiens
ccccuccccacgcucuggaaa

SEQ ID NO: 58 - RNA, 24 nt, Homo sapiens
gcagcaccgggaggcucagacaac

SEQ ID NO: 59 - RNA, 20 nt, Homo sapiens
gagccucaucaaagaaacgg

SEQ ID NO: 60 - RNA, 20 nt, Homo sapiens
gcucccacugggacugagcg

SEQ ID NO: 61 - RNA, 21 nt, Homo sapiens
agaugggaagagagagaagag

SEQ ID NO: 62 - RNA, 30 nt, Homo sapiens
agagacaaggaaaccacacagacagagacc

SEQ ID NO: 63 - RNA, 19 nt, Homo sapiens
gccgcccagcagagagagg

SEQ ID NO: 64 - RNA, 23 nt, Homo sapiens
agcuggcugggcccaccuggcau

SEQ ID NO: 65 - RNA, 18 nt, Homo sapiens
gggcccaggcagaagccu

SEQ ID NO: 66 - RNA, 21 nt, Homo sapiens
uccccagagcuuucaacacag

SEQ ID NO: 67 - RNA, 24 nt, Homo sapiens
gcagccacagcucaaagcugagga

SEQ ID NO: 68 - RNA, 29 nt, Homo sapiens
gaucagacacguaaggaaaacgcauuaua

SEQ ID NO: 69 - RNA, 30 nt, Homo sapiens
gcagaaggcacuaaucaagucaaggucaca

SEQ ID NO: 70 - RNA, 24 nt, Homo sapiens
cgggcauuaaagagcuggacucag

SEQ ID NO: 71 - RNA, 20 nt, Homo sapiens
accaauuuugaaaaaagcag

SEQ ID NO: 72 - RNA, 22 nt, Homo sapiens
ccacauuuuaauuuaauuuuac

SEQ ID NO: 73 - RNA, 19 nt, Homo sapiens
ccauuagaaagaauaaaag

SEQ ID NO: 74 - RNA, 28 nt, Homo sapiens
uauuuuaaauuaauuaaauguuaaaugg

SEQ ID NO: 75 - RNA, 22 nt, Homo sapiens
auuucauuuuaaacucacagau

SEQ ID NO: 76 - RNA, 22 nt, Homo sapiens
auccuugcaaagagaagaaaug

SEQ ID NO: 77 - RNA, 39 nt, Homo sapiens
uccuucaacuugacuucuugcugauggcucagaucaacu

SEQ ID NO: 78 - RNA, 36 nt, Homo sapiens
uauuuuauaaaaguaaaaugccaagaaccaaagacu

SEQ ID NO: 79 - RNA, 34 nt, Homo sapiens
uucaaacuccaagaaauacaaauucucaaaacac

SEQ ID NO: 80 - RNA, 22 nt, Homo sapiens
uuuucucaagacaaagaaaccc

SEQ ID NO: 81 - RNA, 18 nt, Homo sapiens
ggguggagcagucaagcc

SEQ ID NO: 82 - RNA, 24 nt, Homo sapiens
acuucccaacccacacacacagac

SEQ ID NO: 83 - RNA, 22 nt, Homo sapiens
gucacauaaaaaucagaagaau

SEQ ID NO: 84 - RNA, 21 nt, Homo sapiens
caaauauuaucagagauugaa

SEQ ID NO: 85 - RNA, 29 nt, Homo sapiens
cuugaauuauuguuuuuauuuugacaauc

SEQ ID NO: 86 - RNA, 28 nt, Homo sapiens
acucaauaauuaaagauuugggaaauau

SEQ ID NO: 87 - RNA, 22 nt, Homo sapiens
aggcaacauuuaccuugaaaau

SEQ ID NO: 88 - RNA, 22 nt, Homo sapiens
gagggcaaucuucagaauucag

SEQ ID NO: 89 - RNA, 35 nt, Homo sapiens
uaaucagauuugacaguuggcuuucugaaaguuuu

SEQ ID NO: 90 - RNA, 29 nt, Homo sapiens
acauuucuggagaauuauaauaaacuuau

SEQ ID NO: 91 - RNA, 24 nt, Homo sapiens
caauuacacagauucauuuagaua

SEQ ID NO: 92 - RNA, 32 nt, Homo sapiens
ucagauuugcuacuuugaauuuagcacauuau

SEQ ID NO: 93 - RNA, 31 nt, Homo sapiens
aaauaaagcucauuaaucucccauuuucaug

SEQ ID NO: 94 - RNA, 22 nt, Homo sapiens
ugaaaaugaaaaaaauaaaugu

SEQ ID NO: 95 - RNA, 34 nt, Homo sapiens
gcuacaaacacucuguaaauagcuuagaaaaacu

SEQ ID NO: 96 - RNA, 34 nt, Homo sapiens
caugauuucuauaagacagaaauagagcagauaa

SEQ ID NO: 97 - RNA, 29 nt, Homo sapiens
caauuaccaacagauuuucuucaucaaug

SEQ ID NO: 98 - RNA, 22 nt, Homo sapiens
acauaaacuucaaauuaaaccu

SEQ ID NO: 99 - RNA, 25 nt, Homo sapiens
guaccuuugcuuaguuuaaaaauug

SEQ ID NO: 100 - RNA, 23 nt, Homo sapiens
ggaauuugauaauuuucuaaagg

SEQ ID NO: 101 - RNA, 19 nt, Homo sapiens
cggaagggagaaagaaggg

SEQ ID NO: 102 - RNA, 17 nt, Homo sapiens
ccuggccucacucagcg

SEQ ID NO: 103 - RNA, 22 nt, Homo sapiens
uaaagaaauaaugcuuacuggu

SEQ ID NO: 104 - RNA, 22 nt, Homo sapiens
ugugguaaucaaagcaaauaga

SEQ ID NO: 105 - RNA, 31 nt, Homo sapiens
augauuuagaacagcaugaaaaaucaaaaua

SEQ ID NO: 106 - RNA, 24 nt, Homo sapiens
cuuaaauuuaaauuaagaaaugag

SEQ ID NO: 107 - RNA, 27 nt, Homo sapiens
uaaaagaaaauggauucuaauuaauau

SEQ ID NO: 108 - RNA, 29 nt, Homo sapiens
gcaaagccacagcugagggugacagcacg

SEQ ID NO: 109 - RNA, 21 nt, Homo sapiens
ccagccagaggagaaaaggca

SEQ ID NO: 110 - RNA, 24 nt, Homo sapiens
cacacaaauaaagaaauuagauuu

SEQ ID NO: 111 - RNA, 34 nt, Homo sapiens
uuuucuucuuuuauuuucauucuccaauuuuaaa

SEQ ID NO: 112 - RNA, 29 nt, Homo sapiens
aagccaggaaaaagaaaucuuuucuauca

SEQ ID NO: 113 - RNA, 21 nt, Homo sapiens
agaaacacauucaguuucuac

SEQ ID NO: 114 - RNA, 21 nt, Homo sapiens
ucuaaaaaaaaaaauuuucuc

SEQ ID NO: 115 - RNA, 24 nt, Homo sapiens
ugcauaaugcauggcaaaaugagc

SEQ ID NO: 116 - RNA, 32 nt, Homo sapiens
gcuagagaagcuaugacucugaggucaaggac

SEQ ID NO: 117 - RNA, 21 nt, Homo sapiens
cuucaucaaagaaugcaauca

SEQ ID NO: 118 - RNA, 17 nt, Homo sapiens
acuuugaguaaaagaau

SEQ ID NO: 119 - RNA, 25 nt, Homo sapiens
cuuugcuuucucaaguuuuguaugu

SEQ ID NO: 120 - RNA, 26 nt, Homo sapiens
ccagcagaggcaggcagagaaggaag

SEQ ID NO: 121 - RNA, 35 nt, Homo sapiens
cugaaaugagaaacagaagacacauaagagaaccc

SEQ ID NO: 122 - RNA, 26 nt, Homo sapiens
gccgcguacauacacacagaacaacc

SEQ ID NO: 123 - RNA, 57 nt, Homo sapiens
ugagcaucccuugggccucaacccuacucacaucagggaaaggugaaaggguaaacu

SEQ ID NO: 124 - RNA, 24 nt, Homo sapiens
aggcuuagaggaaaaggugagcau

SEQ ID NO: 125 - RNA, 25 nt, Homo sapiens
uauuucaugcucaagaacccaacca

SEQ ID NO: 126 - RNA, 27 nt, Homo sapiens
cacaucagggaaaggugaaaggguaaa

SEQ ID NO: 127 - RNA, 17 nt, Homo sapiens
cccacgccgcccgcccg

SEQ ID NO: 128 - RNA, 28 nt, Homo sapiens
ucugaggcccaggguccagcuguggaug

SEQ ID NO: 129 - RNA, 25 nt, Homo sapiens
cagccauccaagcacaaccacugcu

SEQ ID NO: 130 - RNA, 29 nt, Homo sapiens
cucacugacagaugugagcuggaagcuga

SEQ ID NO: 131 - RNA, 21 nt, Homo sapiens
ggguucuaugugcagacucag

SEQ ID NO: 132 - RNA, 19 nt, Homo sapiens
caucacucacgagaauucc

SEQ ID NO: 133 - RNA, 21 nt, Homo sapiens
acagaccagggaucacccaga

SEQ ID NO: 134 - RNA, 22 nt, Homo sapiens
uuuagauuaaugagauuuuugc

SEQ ID NO: 135 - RNA, 25 nt, Homo sapiens
ugcauuuuucuuuaaagcuauuuug

SEQ ID NO: 136 - RNA, 28 nt, Homo sapiens
aagacccagaagccaucucagaagauug

SEQ ID NO: 137 - RNA, 33 nt, Homo sapiens
augacagggacaaggacaaugaaucagaaguag

SEQ ID NO: 138 - RNA, 28 nt, Homo sapiens
uuuucuuacaacaccaacaggaagaagu

SEQ ID NO: 139 - RNA, 28 nt, Homo sapiens
guuuauguuaccucuuuacacugaaaug

SEQ ID NO: 140 - RNA, 22 nt, Homo sapiens
gggacacagaugaaggaaugag

SEQ ID NO: 141 - RNA, 31 nt, Homo sapiens
caaggaagggaagguggugccagaaagcagg

SEQ ID NO: 142 - RNA, 19 nt, Homo sapiens
aggcuuaugaaacacaacc

SEQ ID NO: 143 - RNA, 21 nt, Homo sapiens
agggccaaagcugccaggagu

SEQ ID NO: 144 - RNA, 30 nt, Homo sapiens
cucccuuucucccccucccuccucugcuca

SEQ ID NO: 145 - RNA, 21 nt, Homo sapiens
cuggagccagggagcagagcg

SEQ ID NO: 146 - RNA, 25 nt, Homo sapiens
cucagcaacaguuucaaguucccac

SEQ ID NO: 147 - RNA, 33 nt, Homo sapiens
ccgccaccaagacugccagcucccacccaccuc

SEQ ID NO: 148 - RNA, 23 nt, Homo sapiens
agugccucagaucccaccagagg

SEQ ID NO: 149 - RNA, 26 nt, Homo sapiens
gccugcuaccagcaacucucauuucc

SEQ ID NO: 150 - RNA, 28 nt, Homo sapiens
cacagagaagaaccuucacugcuucugc

SEQ ID NO: 151 - RNA, 21 nt, Homo sapiens
gaggacacaggcaaaggaggg

SEQ ID NO: 152 - RNA, 21 nt, Homo sapiens
ccaaagcugccaggaguugca

SEQ ID NO: 153 - RNA, 18 nt, Homo sapiens
gcuggaggucaggcuggg

SEQ ID NO: 154 - RNA, 23 nt, Homo sapiens
cccucagcaacaguuucaaguuc

SEQ ID NO: 155 - RNA, 26 nt, Homo sapiens
aauagucugcugugcuggagaaaggg

SEQ ID NO: 156 - RNA, 28 nt, Homo sapiens
uuccuccuagcuggagggauggagaaag

SEQ ID NO: 157 - RNA, 25 nt, Homo sapiens
agagagugccucagaucccaccaga

SEQ ID NO: 158 - RNA, 36 nt, Homo sapiens
agaaggagggagccugcuaccagcaacucucauuuc

SEQ ID NO: 159 - RNA, 21 nt, Homo sapiens
cacacagagaagaaccuucac

SEQ ID NO: 160 - RNA, 23 nt, Homo sapiens
cagcacagaggcaggcacaaaug

SEQ ID NO: 161 - RNA, 21 nt, Homo sapiens
ucuggaacgggagggagaggg

SEQ ID NO: 162 - RNA, 22 nt, Homo sapiens
cucagccagagaccugagcagc

SEQ ID NO: 163 - RNA, 25 nt, Homo sapiens
caauuucaacgaucaguaacagagc

SEQ ID NO: 164 - RNA, 23 nt, Homo sapiens
uucuggaaagcgggauaauggac

SEQ ID NO: 165 - RNA, 27 nt, Homo sapiens
caucauaaaaggaguaacaggauaaua

SEQ ID NO: 166 - RNA, 22 nt, Homo sapiens
cuuauuucagaagaaaauccga

SEQ ID NO: 167 - RNA, 26 nt, Homo sapiens
caagcuuggcauuuuucuuuaaucca

SEQ ID NO: 168 - RNA, 22 nt, Homo sapiens
guggaaacauaaagaaagcauc

SEQ ID NO: 169 - RNA, 27 nt, Homo sapiens
ugcaaaaaaguggaaaaaguaaaugua

SEQ ID NO: 170 - RNA, 27 nt, Homo sapiens
aucuucagguuucuggacucucaccca

SEQ ID NO: 171 - RNA, 22 nt, Homo sapiens
aaacaaaauuagguaaaaggag

SEQ ID NO: 172 - RNA, 21 nt, Homo sapiens
cuuuaaacacaaaaguuuaca

SEQ ID NO: 173 - RNA, 26 nt, Homo sapiens
ggaaaugcagaaauuaauuucuuaug

SEQ ID NO: 174 - RNA, 37 nt, Homo sapiens
auuucaagacaaccauucaaaggcaguuaguuaacaa

SEQ ID NO: 175 - RNA, 26 nt, Homo sapiens
cuaaacaaaguuuucuaaaccagauu

SEQ ID NO: 176 - RNA, 20 nt, Homo sapiens
ggacagaacacacacagaac

SEQ ID NO: 177 - RNA, 27 nt, Homo sapiens
aguuaaaaaucaacuuuaauuuugaag

SEQ ID NO: 178 - RNA, 20 nt, Homo sapiens
uuuuccaaaucagaagauug

SEQ ID NO: 179 - RNA, 25 nt, Homo sapiens
uauuuuaaaacauccaaaaagaagu

SEQ ID NO: 180 - RNA, 25 nt, Homo sapiens
gacaaagcauguuaaaaaguuucca

SEQ ID NO: 181 - RNA, 19 nt, Homo sapiens
aucagaugagcagcagcgg

SEQ ID NO: 182 - RNA, 20 nt, Homo sapiens
gggucaaggcaggcugagag

SEQ ID NO: 183 - RNA, 34 nt, Homo sapiens
ccagaaaccaugagauuugggucagaaaaaggca

SEQ ID NO: 184 - RNA, 21 nt, Homo sapiens
cagucggcgucccagagaucc

SEQ ID NO: 185 - RNA, 23 nt, Homo sapiens
cauuuaaguagcaaauucugggc

SEQ ID NO: 186 - RNA, 20 nt, Homo sapiens
cucaucuucuucagagaagu

SEQ ID NO: 187 - RNA, 22 nt, Homo sapiens
ccaaagaauuggcaaagaaaag

SEQ ID NO: 188 - RNA, 21 nt, Homo sapiens
auuucacuggcauuaagacag

SEQ ID NO: 189 - RNA, 22 nt, Homo sapiens
guccguagcaguuagcagauga

SEQ ID NO: 190 - RNA, 23 nt, Homo sapiens
gucugagucagggccaaaaggaa

SEQ ID NO: 191 - RNA, 25 nt, Homo sapiens
gggaaacagcaugaagauaagcagg

SEQ ID NO: 192 - RNA, 19 nt, Homo sapiens
augagaaacuagauuaggg

SEQ ID NO: 193 - RNA, 26 nt, Homo sapiens
gaaaagcaauaaagaaaugagcaaca

SEQ ID NO: 194 - RNA, 23 nt, Homo sapiens
aaguccagaaaccaguuucaguc

SEQ ID NO: 195 - RNA, 25 nt, Homo sapiens
gagcugggaaaggguugugagagac

SEQ ID NO: 196 - RNA, 20 nt, Homo sapiens
ggucccugaagccugucacc

SEQ ID NO: 197 - RNA, 21 nt, Homo sapiens
cgcuuaaguuguggaaggucg

SEQ ID NO: 198 - RNA, 25 nt, Homo sapiens
agcacuacagggccuccagcagggc

SEQ ID NO: 199 - RNA, 29 nt, Homo sapiens
acaaaaccagacacuucucauggacagca

SEQ ID NO: 200 - RNA, 25 nt, Homo sapiens
aucugaagacaucucuucccacauu

SEQ ID NO: 201 - RNA, 22 nt, Homo sapiens
ccagucaagcauuagauuuagc

SEQ ID NO: 202 - RNA, 18 nt, Homo sapiens
uccuccuucuaaaacauu

SEQ ID NO: 203 - RNA, 17 nt, Homo sapiens
aggaugcaccccaugcu

SEQ ID NO: 204 - RNA, 27 nt, Homo sapiens
cggagccacaagcaauucaaauccagc

SEQ ID NO: 205 - RNA, 28 nt, Homo sapiens
gucagcagucgggacacgguggguuaga

SEQ ID NO: 206 - RNA, 43 nt, Homo sapiens
ugguuaaagaaacuggagaaagaaaagcaaaaggauaaaggaa

SEQ ID NO: 207 - RNA, 25 nt, Homo sapiens
caagucagggagagagagagagagg

SEQ ID NO: 208 - RNA, 21 nt, Homo sapiens
agccgccccgcucuccccagc

SEQ ID NO: 209 - RNA, 19 nt, Homo sapiens
gaggaugaaagaggaaagg

SEQ ID NO: 210 - RNA, 21 nt, Homo sapiens
cugagggcacaagagagacag

SEQ ID NO: 211 - RNA, 23 nt, Homo sapiens
gggaagacaaagacuugacaagg

SEQ ID NO: 212 - RNA, 28 nt, Homo sapiens
aggucaaacagguggucaaacagcagga

SEQ ID NO: 213 - RNA, 20 nt, Homo sapiens
uaaggacugaagacacgacg

SEQ ID NO: 214 - RNA, 25 nt, Homo sapiens
gaguguugaaggcaagacuuugcag

SEQ ID NO: 215 - RNA, 25 nt, Homo sapiens
cccacucagugggagcugcagccau

SEQ ID NO: 216 - RNA, 22 nt, Homo sapiens
ggaagacccauuucuccaugcc

SEQ ID NO: 217 - RNA, 26 nt, Homo sapiens
cccagagcucugagggugcccugggc

SEQ ID NO: 218 - RNA, 18 nt, Homo sapiens
gugcucacccagcaggca

SEQ ID NO: 219 - RNA, 28 nt, Homo sapiens
gccacgugcugacucugcagcuggcagg

SEQ ID NO: 220 - RNA, 18 nt, Homo sapiens
ucgcccccagucuucccu

SEQ ID NO: 221 - RNA, 17 nt, Homo sapiens
ggcagcacagcaagagg

SEQ ID NO: 222 - RNA, 26 nt, Homo sapiens
caaaaacagugcuacacauuuacuca

SEQ ID NO: 223 - RNA, 23 nt, Homo sapiens
ucagaaagccugugacaaaucuu

SEQ ID NO: 224 - RNA, 20 nt, Homo sapiens
aagaagaguccaaaaugguu

SEQ ID NO: 225 - RNA, 29 nt, Homo sapiens
ugagaagaaugaaauaaaauuuaacaaaa

SEQ ID NO: 226 - RNA, 25 nt, Homo sapiens
uguuaugcuaaaaauguaagaaaac

SEQ ID NO: 227 - RNA, 24 nt, Homo sapiens
aucagaauuuccaagagagaggcc

SEQ ID NO: 228 - RNA, 32 nt, Homo sapiens
uaaggaaagaaaacagcauugcaaagaacacg

SEQ ID NO: 229 - RNA, 28 nt, Homo sapiens
aguuuuaaaacuuuucuaaguuuaaugu

SEQ ID NO: 230 - RNA, 20 nt, Homo sapiens
aaugaaaacaugaaaucuga

SEQ ID NO: 231 - RNA, 29 nt, Homo sapiens
gaaaauuugugggaaaaguuuauccuuac

SEQ ID NO: 232 - RNA, 28 nt, Homo sapiens
ucugaaacaguaauucaugcauaauucu

SEQ ID NO: 233 - RNA, 25 nt, Homo sapiens
ugcagaacuucaauuucauaauuuu

SEQ ID NO: 234 - RNA, 29 nt, Homo sapiens
aaacaaaucaagaccaaacuucagagagu

SEQ ID NO: 235 - RNA, 23 nt, Homo sapiens
ccugaaaaugagaauaaaucucc

SEQ ID NO: 236 - RNA, 22 nt, Homo sapiens
gacaaaucaugagauucucacc

SEQ ID NO: 237 - RNA, 18 nt, Homo sapiens
ucccugccacucccucca

SEQ ID NO: 238 - RNA, 21 nt, Homo sapiens
cugcaggaagagaggcagcga

SEQ ID NO: 239 - RNA, 17 nt, Homo sapiens
gccuuuuucauuaaaag

SEQ ID NO: 240 - RNA, 24 nt, Homo sapiens
uuucauuuguuuuuaaacuuagau

SEQ ID NO: 241 - RNA, 17 nt, Homo sapiens
uauucaugaauuucuaa

SEQ ID NO: 242 - RNA, 23 nt, Homo sapiens
uuuccaaauguaaaauaaucaca

SEQ ID NO: 243 - RNA, 21 nt, Homo sapiens
cacaaaacauaaaacauaaac

SEQ ID NO: 244 - RNA, 20 nt, Homo sapiens
uacuaggaagcaaguuauua

SEQ ID NO: 245 - RNA, 19 nt, Homo sapiens
aauucauuauuuaaaugac

SEQ ID NO: 246 - RNA, 24 nt, Homo sapiens
augaaauuuaaaauccacauuagc

SEQ ID NO: 247 - RNA, 18 nt, Homo sapiens
acauucugauuagggagg

SEQ ID NO: 248 - RNA, 23 nt, Homo sapiens
gaaggcaacagaggugaguguga

SEQ ID NO: 249 - RNA, 25 nt, Homo sapiens
ccagagggcaggcaaggcagaagug

SEQ ID NO: 250 - RNA, 21 nt, Homo sapiens
ggaagauuugcaaugguucug

SEQ ID NO: 251 - RNA, 34 nt, Homo sapiens
acacacagacaaaagaguugcaagagacagagac

SEQ ID NO: 252 - RNA, 20 nt, Homo sapiens
ggcaaacuagaauagaaaga

SEQ ID NO: 253 - RNA, 26 nt, Homo sapiens
ccagagcagagagaggguuaaacagg

SEQ ID NO: 254 - RNA, 27 nt, Homo sapiens
ucagcaguagacacacaaauaaaccag

SEQ ID NO: 255 - RNA, 25 nt, Homo sapiens
gucggugccuaauuaucuucuuggg

SEQ ID NO: 256 - RNA, 18 nt, Homo sapiens
aguuuuucagccacuucu

SEQ ID NO: 257 - RNA, 19 nt, Homo sapiens
ucuugcugccuaaaaucac

SEQ ID NO: 258 - RNA, 20 nt, Homo sapiens
ugccuuuacccaaauuccuc

SEQ ID NO: 259 - RNA, 29 nt, Homo sapiens
uucaaggucauuucuacagaccaauuucu

SEQ ID NO: 260 - RNA, 25 nt, Homo sapiens
ggacacuguccaacaaagauucuac

SEQ ID NO: 261 - RNA, 18 nt, Homo sapiens
cuggcaacccagggacac

SEQ ID NO: 262 - RNA, 24 nt, Homo sapiens
aauaaaauugaguuuauagaauua

SEQ ID NO: 263 - RNA, 32 nt, Homo sapiens
auuugccagauuucaauuuaaaguuuaaaaag

SEQ ID NO: 264 - RNA, 35 nt, Homo sapiens
aaacugaaaacacacaaaucuuugaaaugaaaugc

SEQ ID NO: 265 - RNA, 22 nt, Homo sapiens
cuuuuuuauuuuaagaguucca

SEQ ID NO: 266 - RNA, 24 nt, Homo sapiens
augauuuucacaaagagaacaaua

SEQ ID NO: 267 - RNA, 29 nt, Homo sapiens
auuucauaauaaaagcacauaaaauuagu

SEQ ID NO: 268 - RNA, 21 nt, Homo sapiens
ccugccacccaccgcucaccc

SEQ ID NO: 269 - RNA, 20 nt, Homo sapiens
ccuuccuccuccugggacaa

SEQ ID NO: 270 - RNA, 33 nt, Homo sapiens
auuaaagugucagaacuaagaccaaaacagaug

SEQ ID NO: 271 - RNA, 30 nt, Homo sapiens
ccugaaauccuugccucacagaggagaacu

SEQ ID NO: 272 - RNA, 19 nt, Homo sapiens
gccucaguccugaaauccu

SEQ ID NO: 273 - RNA, 22 nt, Homo sapiens
ggcaguaaaacgugccaucuuc

SEQ ID NO: 274 - RNA, 20 nt, Homo sapiens
ugucgcagaccuccugaggg

SEQ ID NO: 275 - RNA, 25 nt, Homo sapiens
ucuuccuuuucccucugcuaaguuu

SEQ ID NO: 276 - RNA, 25 nt, Homo sapiens
gugacuauggaaaauccccuaacag

SEQ ID NO: 277 - RNA, 21 nt, Homo sapiens
gugcagcucugauguggcagg

SEQ ID NO: 278 - RNA, 22 nt, Homo sapiens
ugcagggagugggaaggcagau

SEQ ID NO: 279 - RNA, 28 nt, Homo sapiens
gggccgcagagaccgaagagggcaggug

SEQ ID NO: 280 - RNA, 29 nt, Homo sapiens
gaagccagggcguagcaagguuguagcaa

SEQ ID NO: 281 - RNA, 19 nt, Homo sapiens
gggcaaccugggcacugca

SEQ ID NO: 282 - RNA, 22 nt, Homo sapiens
uuuuuccuucauuuccugggau

SEQ ID NO: 283 - RNA, 23 nt, Homo sapiens
gucccaaacccuaaacuuaccuc

SEQ ID NO: 284 - RNA, 20 nt, Homo sapiens
cugggauucccacagaacgg

SEQ ID NO: 285 - RNA, 26 nt, Homo sapiens
gcuggaaacguccccaguggccuucc

SEQ ID NO: 286 - RNA, 22 nt, Homo sapiens
ggcggagcccucccgcagaggc

SEQ ID NO: 287 - RNA, 22 nt, Homo sapiens
gcagcaggcaagcaauuuauug

SEQ ID NO: 288 - RNA, 23 nt, Homo sapiens
gcccuuggcaacagguuaaggga

SEQ ID NO: 289 - RNA, 22 nt, Homo sapiens
cagguccuggaaacagggccaa

SEQ ID NO: 290 - RNA, 20 nt, Homo sapiens
ggguaagaaaaccagacaua

SEQ ID NO: 291 - RNA, 20 nt, Homo sapiens
gcacauuuaacagaaaaaug

SEQ ID NO: 292 - RNA, 26 nt, Homo sapiens
ugaagacgaagaaaaagccagccagg

SEQ ID NO: 293 - RNA, 21 nt, Homo sapiens
cgcacgcggccggccgcccgc

SEQ ID NO: 294 - RNA, 19 nt, Homo sapiens
ccacccccaaaagcagaau

SEQ ID NO: 295 - RNA, 20 nt, Homo sapiens
cugccccucccagaaugcug

SEQ ID NO: 296 - RNA, 23 nt, Homo sapiens
ucuuucaccuaccagacacagac

SEQ ID NO: 297 - RNA, 22 nt, Homo sapiens
ccuccagagaauguaaagcuga

SEQ ID NO: 298 - RNA, 24 nt, Homo sapiens
ggagagggcuggaaggauguggca

SEQ ID NO: 299 - RNA, 25 nt, Homo sapiens
aaaaacgaagccaucagaugccaag

SEQ ID NO: 300 - RNA, 21 nt, Homo sapiens
gugacaaaugcaaauaaauac

SEQ ID NO: 301 - RNA, 28 nt, Homo sapiens
cugccaacaaagagagaaaauauuagcu

SEQ ID NO: 302 - RNA, 25 nt, Homo sapiens
uguuuggaaaaugagaaauaaaugu

SEQ ID NO: 303 - RNA, 25 nt, Homo sapiens
uagcaaaugugacuagcaaaccaac

SEQ ID NO: 304 - RNA, 29 nt, Homo sapiens
cuaauuacuggaauuuuguuuaaauaauc

SEQ ID NO: 305 - RNA, 28 nt, Homo sapiens
uuguuagcuagagagggugggcaaaggg

SEQ ID NO: 306 - RNA, 20 nt, Homo sapiens
ccuaauccacuauuugaaac

SEQ ID NO: 307 - RNA, 22 nt, Homo sapiens
caugccucacgccauccuaaug

SEQ ID NO: 308 - RNA, 19 nt, Homo sapiens
gacagggacggagcggcgg

SEQ ID NO: 309 - RNA, 19 nt, Homo sapiens
accucccucaccccaaacc

SEQ ID NO: 310 - RNA, 19 nt, Homo sapiens
ggccgcagaggaaaggagg

SEQ ID NO: 311 - RNA, 20 nt, Homo sapiens
gcagccccgugacacaggag

SEQ ID NO: 312 - RNA, 18 nt, Homo sapiens
cacaggccgcgccgcccc

SEQ ID NO: 313 - RNA, 24 nt, Homo sapiens
ccaugcugggccagaucugccagg

SEQ ID NO: 314 - RNA, 22 nt, Homo sapiens
cugagaggucgaagcagaaugc

SEQ ID NO: 315 - RNA, 26 nt, Homo sapiens
gugaaaugaagaccacagucaagccc

SEQ ID NO: 316 - RNA, 27 nt, Homo sapiens
gagacagggcugcaggcaagucaagua

SEQ ID NO: 317 - RNA, 27 nt, Homo sapiens
acacacacaaccaaacacgcacaacac

SEQ ID NO: 318 - RNA, 21 nt, Homo sapiens
ggcagcaggagcagaaaccag

SEQ ID NO: 319 - RNA, 24 nt, Homo sapiens
cacaacagucagcaggucagacug

SEQ ID NO: 320 - RNA, 21 nt, Homo sapiens
gaagggucugggaccgcagca

SEQ ID NO: 321 - RNA, 18 nt, Homo sapiens
uacagugagaaaggcgcu

SEQ ID NO: 322 - RNA, 32 nt, Homo sapiens
aggaacuuaauccaaacccgaagaaggaagac

SEQ ID NO: 323 - RNA, 23 nt, Homo sapiens
ccucuuaaaaguuauuauuuauu

SEQ ID NO: 324 - RNA, 22 nt, Homo sapiens
aauuucaaugagaauaaugaau

SEQ ID NO: 325 - RNA, 21 nt, Homo sapiens
ucuuuaagauaaaguucaaac

SEQ ID NO: 326 - RNA, 21 nt, Homo sapiens
caauuugaaugcacauuugau

SEQ ID NO: 327 - RNA, 20 nt, Homo sapiens
cgacagacguggccaaggca

SEQ ID NO: 328 - RNA, 25 nt, Homo sapiens
agacacagcaaccgaagccaacacu

SEQ ID NO: 329 - RNA, 24 nt, Homo sapiens
acacaggccgcgggcuccacaaac

SEQ ID NO: 330 - RNA, 21 nt, Homo sapiens
gagcuccauuacucuccucau

SEQ ID NO: 331 - RNA, 20 nt, Homo sapiens
caccucccgccaaccauucc

SEQ ID NO: 332 - RNA, 21 nt, Homo sapiens
uuccuucauauuuccagaguc

SEQ ID NO: 333 - RNA, 20 nt, Homo sapiens
uccccagcucugaaaucucu

SEQ ID NO: 334 - RNA, 25 nt, Homo sapiens
cucacacaagcaggagaaaggagau

SEQ ID NO: 335 - RNA, 20 nt, Homo sapiens
cuagucuucagcccacccag

SEQ ID NO: 336 - RNA, 24 nt, Homo sapiens
acaauacuuagaaacacauaaugg

SEQ ID NO: 337 - RNA, 18 nt, Homo sapiens
cguagaauuuaaaccacc

SEQ ID NO: 338 - RNA, 21 nt, Homo sapiens
cacauuauguuaauuaacaac

SEQ ID NO: 339 - RNA, 29 nt, Homo sapiens
agaagaaaaacaaaauuauuuaauaaaau

SEQ ID NO: 340 - RNA, 37 nt, Homo sapiens
uaacugaaaugaauucauucaagaggaaaauauggaa

SEQ ID NO: 341 - RNA, 28 nt, Homo sapiens
ucagaauuacagaguaaggaaaagaccu

SEQ ID NO: 342 - RNA, 29 nt, Homo sapiens
ggcaucacaaaaugacuuuaauuucugga

SEQ ID NO: 343 - RNA, 21 nt, Homo sapiens
cuaaccccagagaggucucua

SEQ ID NO: 344 - RNA, 22 nt, Homo sapiens
uggagacccugggucccugcag

SEQ ID NO: 345 - RNA, 18 nt, Homo sapiens
ccacaggagcucugggcu

SEQ ID NO: 346 - RNA, 22 nt, Homo sapiens
ugggcccaccgccaaagcagcg

SEQ ID NO: 347 - RNA, 27 nt, Homo sapiens
uccacgcccuugaagaggucacggcgg

SEQ ID NO: 348 - RNA, 22 nt, Homo sapiens
auuucucucuuuuaaaaagcug

SEQ ID NO: 349 - RNA, 23 nt, Homo sapiens
gcacaaaagaaaagaccaaaagu

SEQ ID NO: 350 - RNA, 27 nt, Homo sapiens
cagaagucaaaaagauuuggaggaaag

SEQ ID NO: 351 - RNA, 22 nt, Homo sapiens
aaaccucagaagucaaaaagau

SEQ ID NO: 352 - RNA, 19 nt, Homo sapiens
uaugacaauccaaacaggc

SEQ ID NO: 353 - RNA, 31 nt, Homo sapiens
uaagaaagggcgcucccacaugcucuuuagg

SEQ ID NO: 354 - RNA, 24 nt, Homo sapiens
uccuaaaauaucuugacaagcaau

SEQ ID NO: 355 - RNA, 25 nt, Homo sapiens
aagcucacauuacagggaagaggga

SEQ ID NO: 356 - RNA, 23 nt, Homo sapiens
ucauuuuauuaacaagaagaguc

SEQ ID NO: 357 - RNA, 25 nt, Homo sapiens
accaagaacugaauucuauuucagg

SEQ ID NO: 358 - RNA, 29 nt, Homo sapiens
gaaacacgggcaaccaugcaagagagacu

SEQ ID NO: 359 - RNA, 22 nt, Homo sapiens
cccaccaggacugaccccuccc

SEQ ID NO: 360 - RNA, 25 nt, Homo sapiens
cccuccugcugcuggaagcaggucc

SEQ ID NO: 361 - RNA, 24 nt, Homo sapiens
gucacagaaaugugaaaaugcacc

SEQ ID NO: 362 - RNA, 21 nt, Homo sapiens
uucuuuaggaagcaggacuga

SEQ ID NO: 363 - RNA, 22 nt, Homo sapiens
gacucagccccagcaaauccgc

SEQ ID NO: 364 - RNA, 18 nt, Homo sapiens
gcacccggcuccggcccc

SEQ ID NO: 365 - RNA, 29 nt, Homo sapiens
gcaaaucacacucccucugaguuggaagc

SEQ ID NO: 366 - RNA, 37 nt, Homo sapiens
ccgccuccagaccgaucccacccggaacacagauggg

SEQ ID NO: 367 - RNA, 21 nt, Homo sapiens
auaccgaagagaagcagggac

SEQ ID NO: 368 - RNA, 26 nt, Homo sapiens
cccagagggaaaagcaaaagcugagg

SEQ ID NO: 369 - RNA, 22 nt, Homo sapiens
gcagacaggcucacguuucucu

SEQ ID NO: 370 - RNA, 22 nt, Homo sapiens
cccagacaagaacucuccucag

SEQ ID NO: 371 - RNA, 17 nt, Homo sapiens
gcugggccucagcagga

SEQ ID NO: 372 - RNA, 24 nt, Homo sapiens
cuuacugaggcuggcacgaagacc

SEQ ID NO: 373 - RNA, 21 nt, Homo sapiens
ccuuaaguuuaaaaauacuga

SEQ ID NO: 374 - RNA, 28 nt, Homo sapiens
aaauguuucuaaauuauucauaaagaug

SEQ ID NO: 375 - RNA, 32 nt, Homo sapiens
aauacuuucauauuuuuauuuacuuuaccucc

SEQ ID NO: 376 - RNA, 28 nt, Homo sapiens
ucuuuaauaagaaaauacauggaacaca

SEQ ID NO: 377 - RNA, 29 nt, Homo sapiens
uauucuauauuuuaauucuaagauacucu

SEQ ID NO: 378 - RNA, 43 nt, Homo sapiens
ugaaagacagacuuuuuucaacacuaccuuaaaaacuuaagac

SEQ ID NO: 379 - RNA, 25 nt, Homo sapiens
aagaucuaauuuuacuauuaagcac

SEQ ID NO: 380 - RNA, 32 nt, Homo sapiens
uauuuguuuccuuuaaagauuuuauaaaagcu

SEQ ID NO: 381 - RNA, 18 nt, Homo sapiens
ccugccaacagcaacugc

SEQ ID NO: 382 - RNA, 21 nt, Homo sapiens
acgugcugggaaccagccagc

SEQ ID NO: 383 - RNA, 23 nt, Homo sapiens
uccgcccccauccacaggagaug

SEQ ID NO: 384 - RNA, 27 nt, Homo sapiens
ggcuuaggguuaggcucaucugaggau

SEQ ID NO: 385 - RNA, 28 nt, Homo sapiens
cugaaauaacuagaguucuaagacacga

SEQ ID NO: 386 - RNA, 36 nt, Homo sapiens
caggaccugccgccagccucggccaggcaggcacgg

SEQ ID NO: 387 - RNA, 21 nt, Homo sapiens
ccacagaagcccuacagcucc

SEQ ID NO: 388 - RNA, 22 nt, Homo sapiens
cggugcagcggucccagagucc

SEQ ID NO: 389 - RNA, 22 nt, Homo sapiens
aggcuuguccaucaaagaaauc

SEQ ID NO: 390 - RNA, 23 nt, Homo sapiens
agggcgaaaggaaaggaaggaug

SEQ ID NO: 391 - RNA, 22 nt, Homo sapiens
agccccacuuccucagaacagg

SEQ ID NO: 392 - RNA, 35 nt, Homo sapiens
ggaaaagagaaagagacaggagaaaacaagagggu

SEQ ID NO: 393 - RNA, 25 nt, Homo sapiens
aacuugagaguacagaaaaagcagg

SEQ ID NO: 394 - RNA, 21 nt, Homo sapiens
ccaguggccagguuuucuaga

SEQ ID NO: 395 - RNA, 21 nt, Homo sapiens
acgaacagauuagaaauaacu

SEQ ID NO: 396 - RNA, 27 nt, Homo sapiens
cuguagaaaauguaaagaagagaaagc

SEQ ID NO: 397 - RNA, 21 nt, Homo sapiens
uagaauucagacaggaaaggg

SEQ ID NO: 398 - RNA, 28 nt, Homo sapiens
caaaccaugcaaagaggaggaagagaaa

SEQ ID NO: 399 - RNA, 18 nt, Homo sapiens
ccuccagacccucaaagc

SEQ ID NO: 400 - RNA, 17 nt, Homo sapiens
ccgccuggcugggaggg

SEQ ID NO: 401 - RNA, 18 nt, Homo sapiens
agcagccccagccccugg

SEQ ID NO: 402 - RNA, 18 nt, Homo sapiens
ccccacccacagugccag

SEQ ID NO: 403 - RNA, 20 nt, Homo sapiens
cucagggauccgacgcagag

SEQ ID NO: 404 - RNA, 22 nt, Homo sapiens
uguuugaaugcggaagucaucc

SEQ ID NO: 405 - RNA, 21 nt, Homo sapiens
auccucaggcagcuuucaacc

SEQ ID NO: 406 - RNA, 19 nt, Homo sapiens
ugaucucagccucaccuag

SEQ ID NO: 407 - RNA, 29 nt, Homo sapiens
cacagauuuaugauaauaagaaaccauua

SEQ ID NO: 408 - RNA, 22 nt, Homo sapiens
cuucuaauucuagaugacauag

SEQ ID NO: 409 - RNA, 25 nt, Homo sapiens
gccgcuuccguuuaauaaaagcauc

SEQ ID NO: 410 - RNA, 20 nt, Homo sapiens
cugguagaaagagacugagc

SEQ ID NO: 411 - RNA, 23 nt, Homo sapiens
cuuaguggcaagaugcauaaaag

SEQ ID NO: 412 - RNA, 24 nt, Homo sapiens
ugcaaaauuuggaaauuguuuuaa

SEQ ID NO: 413 - RNA, 27 nt, Homo sapiens
cacuuaaacagauauacaaagugugaa

SEQ ID NO: 414 - RNA, 20 nt, Homo sapiens
ugacagcugaaguuccacaa

SEQ ID NO: 415 - RNA, 20 nt, Homo sapiens
auggaacaaguccuucacau

SEQ ID NO: 416 - RNA, 26 nt, Homo sapiens
uucaggaaagacaacaaauauaaaca

SEQ ID NO: 417 - RNA, 23 nt, Homo sapiens
uauuugacauuuaauuuaauaca

SEQ ID NO: 418 - RNA, 27 nt, Homo sapiens
uaauuuucucugaacuucuaaaacagu

SEQ ID NO: 419 - RNA, 27 nt, Homo sapiens
caacuaacaaauaauagaaaaauccaa

SEQ ID NO: 420 - RNA, 28 nt, Homo sapiens
uuaauuucauuuauauuauaaaucaugu

SEQ ID NO: 421 - RNA, 27 nt, Homo sapiens
gacagacaagaauguuaaacagaaaua

SEQ ID NO: 422 - RNA, 28 nt, Homo sapiens
gaagcucugcaagaauuccagcaugcac

SEQ ID NO: 423 - RNA, 22 nt, Homo sapiens
ggaaacagaugcuacauaaauc

SEQ ID NO: 424 - RNA, 29 nt, Homo sapiens
gagcaagggccugagauuuugcaagcaug

SEQ ID NO: 425 - RNA, 30 nt, Homo sapiens
cuucagaugcaacccugacaagggacuaau

SEQ ID NO: 426 - RNA, 21 nt, Homo sapiens
gccccugcccuuucugucuca

SEQ ID NO: 427 - RNA, 28 nt, Homo sapiens
guuaaaacauagguuauaaaagaagaac

SEQ ID NO: 428 - RNA, 25 nt, Homo sapiens
uagaagaaagcaaaacaacaaaacu

SEQ ID NO: 429 - RNA, 19 nt, Homo sapiens
aguaaaccaaaaauaaugg

SEQ ID NO: 430 - RNA, 25 nt, Homo sapiens
uuugagaaaaaaaugcaauugacaa

SEQ ID NO: 431 - RNA, 23 nt, Homo sapiens
auucugucccaggaccuaggagu

SEQ ID NO: 432 - RNA, 29 nt, Homo sapiens
ugcagagcagcuugucuuucuucugagag

SEQ ID NO: 433 - RNA, 31 nt, Homo sapiens
uacucacggcucgugucuucagaagccaagg

SEQ ID NO: 434 - RNA, 25 nt, Homo sapiens
ccuuccccacucaggucagcugcua

SEQ ID NO: 435 - RNA, 16 nt, Artificial Sequence
  SSO
agcuggggccuggggu

SEQ ID NO: 436 - RNA, 21 nt, Artificial Sequence
  SSO
ugcagagcuggggccuggggu

SEQ ID NO: 437 - RNA, 20 nt, Artificial Sequence
  SSO
caugcuucacgagcccagcc

SEQ ID NO: 438 - RNA, 17 nt, Artificial Sequence
  SSO
aaggcugcggcuggguc

SEQ ID NO: 439 - RNA, 21 nt, Artificial Sequence
  SSO
ugguagagggagcagaugcug

SEQ ID NO: 440 - RNA, 20 nt, Artificial Sequence
  SSO
ugguacagcauuguuccaca

SEQ ID NO: 441 - RNA, 19 nt, Artificial Sequence
  SSO
cgcacacuagguagagagc

SEQ ID NO: 442 - RNA, 19 nt, Artificial Sequence
  SSO
gaugcagccuguccuggag

SEQ ID NO: 443 - RNA, 21 nt, Artificial Sequence
  SSO
gagcccaccugacgcaaaggc

SEQ ID NO: 444 - RNA, 19 nt, Artificial Sequence
  SSO
uggagggcugagggcugcu

SEQ ID NO: 445 - RNA, 18 nt, Artificial Sequence
  SSO
auggccucuucugaugca

SEQ ID NO: 446 - RNA, 17 nt, Artificial Sequence
  SSO
ucacccccacaugcuuc

SEQ ID NO: 447 - RNA, 14 nt, Artificial Sequence
  SSO
acaugcuucacgag

SEQ ID NO: 448 - RNA, 14 nt, Artificial Sequence
  SSO
cuggggccuggggu

SEQ ID NO: 449 - RNA, 16 nt, Artificial Sequence
  SSO
ugcagagcuggggccu

SEQ ID NO: 450 - RNA, 16 nt, Artificial Sequence
  SSO
aggugcucgcgggugg

SEQ ID NO: 451 - RNA, 21 nt, Artificial Sequence
  SSO
ggguggaagcguccggucgug

SEQ ID NO: 452 - RNA, 20 nt, Artificial Sequence
  SSO
acacacugugccucgccagc

SEQ ID NO: 453 - RNA, 20 nt, Artificial Sequence
  SSO
gacucacuugccguaguuaa

SEQ ID NO: 454 - RNA, 19 nt, Artificial Sequence
  SSO
cacgcucaguagagaaggc

SEQ ID NO: 455 - RNA, 30 nt, Homo sapiens
ggauuccaggguggcuggaccccaggcccc

SEQ ID NO: 456 - RNA, 18 nt, Homo sapiens
ggauuccaggguggcugg

SEQ ID NO: 457 - RNA, 30 nt, Homo sapiens
ggauuccaggguggcugcacgccaggcccc

SEQ ID NO: 458 - RNA, 30 nt, Homo sapiens
ggauuccaggguggcuggacccgaggcgcc

SEQ ID NO: 459 - RNA, 30 nt, Homo sapiens
ggauuccaggaugguaggacccgaggcgcc

SEQ ID NO: 460 - RNA, 30 nt, Homo sapiens
ggauuccaggaugguaggaccccaggcccc

SEQ ID NO: 461 - RNA, 30 nt, Homo sapiens
ggauuccaggguugcuggaccccagucccc

SEQ ID NO: 462 - RNA, 30 nt, Homo sapiens
ggauuccaggguugcuggacccgagucgcc

SEQ ID NO: 463 - DNA, 36 bp, Homo sapiens
attaatacgactcactatagggctcagggttccagg

SEQ ID NO: 464 - DNA, 16 bp, Homo sapiens
tgcagcagggaggacg

SEQ ID NO: 465 - DNA, 15 bp, Homo sapiens
aaatagaggccccag

SEQ ID NO: 466 - DNA, 46 bp, Homo sapiens
gggtggctggaccccaggccccagctctgcagcagggaggacgtgg

SEQ ID NO: 467 - RNA, 30 nt, Homo sapiens
gaagcguggcauuguggaacaaugcuguac

SEQ ID NO: 468 - DNA, 61 bp, Homo sapiens
  misc_feature (4)..(4): A or G
aggrttccagggtggctggaccccaggccccagctctgcagcagggaggacgtggctgggc

SEQ ID NO: 469 - RNA, 19 nt, Homo sapiens
agggaggacguggcugggc

SEQ ID NO: 470 - RNA, 20 nt, Homo sapiens
aggauuccaggguggcugga

SEQ ID NO: 471 - RNA, 20 nt, Homo sapiens
aggauuccagcguggcugga

SEQ ID NO: 472 - RNA, 22 nt, Homo sapiens
ccaggguggcuggaccccaggc

SEQ ID NO: 473 - RNA, 22 nt, Homo sapiens
ccaggguggcuggacuucaggc